European Patent Application EP 4 814 104 A1, published September 30, 2026. Title: 락토바실러스 플란타럼 WiKim0175을 포함하는 골 관절염 질환의 예방, 개선 또는 치료용 조성물. Applicant: 한국식품연구원. Application KR. The sequence listing filed with the application follows.

SEQUENCE LISTING (1 sequence)

SEQ ID NO: 1 - DNA, 1409 bp, Unknown
  source 1..1409: mol_type = other DNA
tcaggacgaacgctggcggcgtgcctaatacatgcaagtcgaacgaactctggtattgattggtgcttgcatcatgatttacatttgagtgagtggcgaactggtgagtaacacgtgggaaacctgcccagaagcgggggataacacctggaaacagatgctaataccgcataacaacttggaccgcatggtccgagcttgaaagatggcttcggctatcacttttggatggtcccgcggcgtattagctagatggtggggtaacggctcaccatggcaatgatacgtagccgacctgagagggtaatcggccacattgggactgagacacggcccaaactcctacgggaggcagcagtagggaatcttccacaatggacgaaagtctgatggagcaacgccgcgtgagtgaagaagggtttcggctcgtaaaactctgttgttaaagaagaacatatctgagagtaactgttcaggtattgacggtatttaaccagaaagccacggctaactacgtgccagcagccgcggtaatacgtaggtggcaagcgttgtccggatttattgggcgtaaagcgagcgcaggcggttttttaagtctgatgtgaaagccttcggctcaaccgaagaagtgcatcggaaactgggaaacttgagtgcagaagaggacagtggaactccatgtgtagcggtgaaatgcgtagatatatggaagaacaccagtggcgaaggcggctgtctggtctgtaactgacgctgaggctcgaaagtatgggtagcaaacaggattagataccctggtagtccataccgtaaacgatgaatgctaagtgttggagggtttccgcccttcagtgctgcagctaacgcattaagcattccgcctggggagtacggccgcaaggctgaaactcaaaggaattgacgggggcccgcacaagcggtggagcatgtggtttaattcgaagctacgcgaagaaccttaccaggtcttgacatactatgcaaatctaagagattagacgttcccttcggggacatggatacaggtggtgcatggttgtcgtcagctcgtgtcgtgagatgttgggttaagtcccgcaacgagcgcaacccttattatcagttgccagcattaagttgggcactctggtgagactgccggtgacaaaccggaggaaggtggggatgacgtcaaatcatcatgccccttatgacctgggctacacacgtgctacaatggatggtacaacgagttgcgaactcgcgagagtaagctaatctcttaaagccattctcagttcggattgtaggctgcaactcgcctacatgaagtcggaatcgctagtaatcgcggatcagcatgccgcggtgaatacgttcccgggccttgtacacaccgcccgtca